European Patent Specification EP 3 523 449 B1, published August 13, 2025. Title: PHI6 INTERNAL CONTROL COMPOSITIONS, DEVICES & METHODS. Applicant: Roche Diagnostics GmbH F. Hoffmann-La Roche AG Roche Molecular Systems, Inc. The sequence listing filed with the application follows.

SEQUENCE LISTING (3 sequences)

SEQ ID NO: 1 - DNA, 24 bp, Artificial Sequence
  source: /note="Description of Artificial Sequence: Synthetic probe"
tgcgatccgtgtccaagggttcgc

SEQ ID NO: 2 - DNA, 20 bp, Artificial Sequence
  source: /note="Description of Artificial Sequence: Synthetic primer"
gcatttctggagcagtgcat

SEQ ID NO: 3 - DNA, 19 bp, Artificial Sequence
  source: /note="Description of Artificial Sequence: Synthetic primer"
gactgccaaggtgccatta